European Patent Application EP 4 275 757 A2, published November 15, 2023. Title: ATF5 PEPTIDE VARIANTS AND USES THEREOF. Applicant: SAPIENCE THERAPEUTICS, INC. The sequence listing filed with the application follows.

SEQUENCE LISTING (87 sequences)

SEQ ID NO: 1 - protein, 76 aa, synthetic construct
  REGION 1..76: note = Description of Artificial Sequence: Synthetic polypeptide
LEQRAEELARENEELLEKEAEELEQENAELEGECQGLEARNRELRERAESVEREIQYVKDLLIEVYKARSQRTRSA

SEQ ID NO: 2 - protein, 67 aa, synthetic construct
  REGION 1..67: note = Description of Artificial Sequence: Synthetic polypeptide
RQIKIWFQNRRMKWKKLEQRAEELARENEELLEKEAEELEQENAELEGECQGLEARNRELRERAESV

SEQ ID NO: 3 - protein, 38 aa, synthetic construct
  REGION 1..38: note = Description of Artificial Sequence: Synthetic polypeptide
RQIKIWFQNRRMKWKKLEGECQGLEARNRELKERAESV

SEQ ID NO: 4 - protein, 38 aa, synthetic construct
  REGION 1..38: note = Description of Artificial Sequence: Synthetic polypeptide
RQIKIWFQNRRMKWKKLEGEGQGLEARNRELKERAESV

SEQ ID NO: 5 - protein, 38 aa, synthetic construct
  REGION 1..38: note = Description of Artificial Sequence: Synthetic polypeptide
RQIKIWFQNRRMKWKKLEGEAQGLEARNRELKERAESV

SEQ ID NO: 6 - protein, 38 aa, synthetic construct
  REGION 1..38: note = Description of Artificial Sequence: Synthetic polypeptide
RQIKIWFQNRRMKWKKLEGECQGLEARNRELKERAEAV

SEQ ID NO: 7 - protein, 38 aa, synthetic construct
  REGION 1..38: note = Description of Artificial Sequence: Synthetic polypeptide
RQIKIWFQNRRMKWKKLEGECQGLEARLRELKERAESV

SEQ ID NO: 8 - protein, 38 aa, synthetic construct
  REGION 1..38: note = Description of Artificial Sequence: Synthetic polypeptide
RQIKIWFQNRRMKWKKLEGECAGLEARNRELKERAESV

SEQ ID NO: 9 - protein, 38 aa, synthetic construct
  REGION 1..38: note = Description of Artificial Sequence: Synthetic polypeptide
RQIKIWFQNRRMKWKKLEGRCQGLRAENRELEERAESV

SEQ ID NO: 10 - protein, 38 aa, synthetic construct
  REGION 1..38: note = Description of Artificial Sequence: Synthetic polypeptide
RQIKIWFQNRRMKWKKLEGRCQGLRAELRELEERAEAV

SEQ ID NO: 11 - protein, 38 aa, synthetic construct
  REGION 1..38: note = Description of Artificial Sequence: Synthetic polypeptide
RQIKIWFQNRRMKWKKLEGRAQGLRAELRELEERAEAV

SEQ ID NO: 12 - protein, 38 aa, synthetic construct
  REGION 1..38: note = Description of Artificial Sequence: Synthetic polypeptide
RQIKIWFQNRRMKWKKLEGRAAGLRAELRELEERAEAV

SEQ ID NO: 13 - protein, 38 aa, synthetic construct
  REGION 1..38: note = Description of Artificial Sequence: Synthetic polypeptide
  SITE 1: note = D-valine
  SITE 2: note = D-alanine
  SITE 3: note = D-glutamic acid
  SITE 4: note = D-alanine
  SITE 5: note = D-arginine
  SITE 6: note = D-glutamic acid
  SITE 7: note = D-glutamic acid
  SITE 8: note = D-leucine
  SITE 9: note = D-glutamic acid
  SITE 10: note = D-arginine
  SITE 11: note = D-leucine
  SITE 12: note = D-glutamic acid
  SITE 13: note = D-alanine
  SITE 14: note = D-arginine
  SITE 15: note = D-leucine
  SITE 16: note = D-glycine
  SITE 17: note = D-glutamine
  SITE 18: note = D-alanine
  SITE 19: note = D-arginine
  SITE 20: note = D-glycine
  SITE 21: note = D-glutamic acid
  SITE 22: note = D-leucine
  SITE 23: note = D-lysine
  SITE 24: note = D-lysine
  SITE 25: note = D-tryptophan
  SITE 26: note = D-lysine
  SITE 27: note = D-methionine
  SITE 28: note = D-arginine
  SITE 29: note = D-arginine
  SITE 30: note = D-asparagine
  SITE 31: note = D-glutamine
  SITE 32: note = D-phenylalanine
  SITE 33: note = D-tryptophan
  SITE 34: note = D-isoleucine
  SITE 35: note = D-lysine
  SITE 36: note = D-isoleucine
  SITE 37: note = D-glutamine
  SITE 38: note = D-arginine
VAEAREELERLEARLGQARGELKKWKMRRNQFWIKIQR

SEQ ID NO: 14 - protein, 38 aa, synthetic construct
  REGION 1..38: note = Description of Artificial Sequence: Synthetic polypeptide
  SITE 1: note = D-valine
  SITE 2: note = D-alanine
  SITE 3: note = D-glutamic acid
  SITE 4: note = D-alanine
  SITE 5: note = D-arginine
  SITE 6: note = D-glutamic acid
  SITE 7: note = D-glutamic acid
  SITE 8: note = D-leucine
  SITE 9: note = D-glutamic acid
  SITE 10: note = D-arginine
  SITE 11: note = D-leucine
  SITE 12: note = D-glutamic acid
  SITE 13: note = D-alanine
  SITE 14: note = D-arginine
  SITE 15: note = D-leucine
  SITE 16: note = D-glycine
  SITE 17: note = D-glutamine
  SITE 18: note = D-alanine
  SITE 19: note = D-arginine
  SITE 20: note = D-glycine
  SITE 21: note = D-glutamic acid
  SITE 22: note = D-leucine
  SITE 23: note = D-lysine
  SITE 24: note = D-lysine
  SITE 25: note = D-tryptophan
  SITE 26: note = D-lysine
  SITE 27: note = D-methionine
  SITE 28: note = D-arginine
  SITE 29: note = D-arginine
  SITE 30: note = D-asparagine
  SITE 31: note = D-glutamine
  SITE 32: note = D-phenylalanine
  SITE 33: note = D-tryptophan
  SITE 34: note = D-leucine
  SITE 35: note = D-lysine
  SITE 36: note = D-leucine
  SITE 37: note = D-glutamine
  SITE 38: note = D-arginine
VAEAREELERLEARLGQARGELKKWKMRRNQFWLKLQR

SEQ ID NO: 15 - protein, 7 aa, synthetic construct
  REGION 1..7: note = Description of Artificial Sequence: Synthetic peptide
FKKFRKF

SEQ ID NO: 16 - protein, 23 aa, synthetic construct
  REGION 1..23: note = Description of Artificial Sequence: Synthetic peptide
LIRLWSHLIHIWFQNRRLKWKKK

SEQ ID NO: 17 - protein, 27 aa, synthetic construct
  REGION 1..27: note = Description of Artificial Sequence: Synthetic peptide
GALFLGWLGAAGSTMGAWSQPKKKRKV

SEQ ID NO: 18 - protein, 16 aa, synthetic construct
  REGION 1..16: note = Description of Artificial Sequence: Synthetic peptide
AAVALLPAVLLALLAP

SEQ ID NO: 19 - protein, 8 aa, synthetic construct
  REGION 1..8: note = Description of Artificial Sequence: Synthetic peptide
ERKKRRRE

SEQ ID NO: 20 - protein, 22 aa, synthetic construct
  REGION 1..22: note = Description of Artificial Sequence: Synthetic peptide
LGTYTQDFNKTFPQTAIGVGAP

SEQ ID NO: 21 - protein, 18 aa, synthetic construct
  REGION 1..18: note = Description of Artificial Sequence: Synthetic peptide
KLALKLALKALKAALKLA

SEQ ID NO: 22 - protein, 27 aa, synthetic construct
  REGION 1..27: note = Description of Artificial Sequence: Synthetic peptide
GLAFLGFLGAAGSTMGAWSQPKKKRKV

SEQ ID NO: 23 - protein, 10 aa, synthetic construct
  REGION 1..10: note = Description of Artificial Sequence: Synthetic peptide
VQRKRQKLMP

SEQ ID NO: 24 - protein, 8 aa, synthetic construct
  REGION 1..8: note = Description of Artificial Sequence: Synthetic peptide
GRKRKKRT

SEQ ID NO: 25 - protein, 16 aa, synthetic construct
  REGION 1..16: note = Description of Artificial Sequence: Synthetic peptide
RQIKIWFQNRRMKWKK

SEQ ID NO: 26 - protein, 16 aa, synthetic construct
  REGION 1..16: note = Description of Artificial Sequence: Synthetic peptide
RQLKLWFQNRRMKWKK

SEQ ID NO: 27 - protein, 16 aa, synthetic construct
  REGION 1..16: note = Description of Artificial Sequence: Synthetic peptide
REIKIWFQNRRMKWKK

SEQ ID NO: 28 - protein, 20 aa, synthetic construct
  REGION 1..20: note = Description of Artificial Sequence: Synthetic peptide
KETWWETWWTEWSQPKKRKV

SEQ ID NO: 29 - protein, 16 aa, synthetic construct
  REGION 1..16: note = Description of Artificial Sequence: Synthetic peptide
PVIRVWFQNKRCKDKK

SEQ ID NO: 30 - protein, 12 aa, synthetic construct
  REGION 1..12: note = Description of Artificial Sequence: Synthetic peptide
  REGION 7..12: note = This region may encompass 1-6 residues
RRRRRRRRRRRR

SEQ ID NO: 31 - protein, 16 aa, synthetic construct
  REGION 1..16: note = Description of Artificial Sequence: Synthetic peptide
LLIILRRRIRKQAHAH

SEQ ID NO: 32 - protein, 16 aa, synthetic construct
  REGION 1..16: note = Description of Artificial Sequence: Synthetic peptide
RRLRRLLRRLLRRLRR

SEQ ID NO: 33 - protein, 12 aa, synthetic construct
  REGION 1..12: note = Description of Artificial Sequence: Synthetic peptide
RVGRRRRRRRRR

SEQ ID NO: 34 - protein, 9 aa, synthetic construct
  REGION 1..9: note = Description of Artificial Sequence: Synthetic peptide
RRWWRRWRR

SEQ ID NO: 35 - protein, 27 aa, synthetic construct
  REGION 1..27: note = Description of Artificial Sequence: Synthetic peptide
MGLGLHLLVLAAALQGAWSQPKKKRKV

SEQ ID NO: 36 - protein, 7 aa, synthetic construct
  REGION 1..7: note = Description of Artificial Sequence: Synthetic peptide
PKKKRKV

SEQ ID NO: 37 - protein, 18 aa, synthetic construct
  REGION 1..18: note = Description of Artificial Sequence: Synthetic peptide
RGGRLSYSRRRFSTSTGR

SEQ ID NO: 38 - protein, 10 aa, synthetic construct
  REGION 1..10: note = Description of Artificial Sequence: Synthetic peptide
RRLSYSRRRF

SEQ ID NO: 39 - protein, 17 aa, synthetic construct
  REGION 1..17: note = Description of Artificial Sequence: Synthetic peptide
RGGRLAYLRRRWAVLGR

SEQ ID NO: 40 - protein, 11 aa, synthetic construct
  REGION 1..11: note = Description of Artificial Sequence: Synthetic peptide
YGRKKRRQRRR

SEQ ID NO: 41 - protein, 10 aa, synthetic construct
  REGION 1..10: note = Description of Artificial Sequence: Synthetic peptide
YGRKKRRQRR

SEQ ID NO: 42 - protein, 9 aa, synthetic construct
  REGION 1..9: note = Description of Artificial Sequence: Synthetic peptide
GRKKRRQRR

SEQ ID NO: 43 - protein, 13 aa, synthetic construct
  REGION 1..13: note = Description of Artificial Sequence: Synthetic peptide
GRKKRRQRRRPPQ

SEQ ID NO: 44 - protein, 11 aa, synthetic construct
  REGION 1..11: note = Description of Artificial Sequence: Synthetic peptide
GKKKKRKREKL

SEQ ID NO: 45 - protein, 8 aa, synthetic construct
  REGION 1..8: note = Description of Artificial Sequence: Synthetic peptide
SKKKKTKV

SEQ ID NO: 46 - protein, 27 aa, synthetic construct
  REGION 1..27: note = Description of Artificial Sequence: Synthetic peptide
GWTLNSAGYLLGKINLKALAALAKKIL

SEQ ID NO: 47 - protein, 21 aa, synthetic construct
  REGION 1..21: note = Description of Artificial Sequence: Synthetic peptide
AGYLLGKINLKALAALAKKIL

SEQ ID NO: 48 - protein, 12 aa, synthetic construct
  REGION 1..12: note = Description of Artificial Sequence: Synthetic peptide
PLIYLRLLRGQF

SEQ ID NO: 49 - protein, 34 aa, synthetic construct
  REGION 1..34: note = Description of Artificial Sequence: Synthetic polypeptide
DAATATRGRSAASRPTQRPRAPARSASRPRRPVQ

SEQ ID NO: 50 - protein, 16 aa, synthetic construct
  REGION 1..16: note = Description of Artificial Sequence: Synthetic peptide
  SITE 1: note = D-lysine
  SITE 2: note = D-lysine
  SITE 3: note = D-tryptophan
  SITE 4: note = D-lysine
  SITE 5: note = D-methionine
  SITE 6: note = D-arginine
  SITE 7: note = D-arginine
  SITE 8: note = D-asparagine
  SITE 9: note = D-glutamine
  SITE 10: note = D-phenylalanine
  SITE 11: note = D-tryptophan
  SITE 12: note = D-isoleucine
  SITE 13: note = D-lysine
  SITE 14: note = D-isoleucine
  SITE 15: note = D-glutamine
  SITE 16: note = D-arginine
KKWKMRRNQFWIKIQR

SEQ ID NO: 51 - protein, 16 aa, synthetic construct
  REGION 1..16: note = Description of Artificial Sequence: Synthetic peptide
  SITE 1: note = D-lysine
  SITE 2: note = D-lysine
  SITE 3: note = D-tryptophan
  SITE 4: note = D-lysine
  SITE 5: note = D-methionine
  SITE 6: note = D-arginine
  SITE 7: note = D-arginine
  SITE 8: note = D-asparagine
  SITE 9: note = D-glutamine
  SITE 10: note = D-phenylalanine
  SITE 11: note = D-tryptophan
  SITE 12: note = D-leucine
  SITE 13: note = D-lysine
  SITE 14: note = D-leucine
  SITE 15: note = D-glutamine
  SITE 16: note = D-arginine
KKWKMRRNQFWLKLQR

SEQ ID NO: 52 - skipped

SEQ ID NO: 53 - protein, 22 aa, synthetic construct
  REGION 1..22: note = Description of Artificial Sequence: Synthetic peptide
  VARIANT 4: note = E or any positively charged amino acid
  VARIANT 5: note = C or any non-polar amino acid
  VARIANT 6: note = Q or A
  VARIANT 9: note = E or any positively charged amino acid
  VARIANT 11: note = R or any negatively charged amino acid
  VARIANT 12: note = N or any non-polar amino acid
  VARIANT 16: note = K or any negatively charged amino acid
  VARIANT 21: note = S or A
LEGXXXGLXAXXRELXERAEXV

SEQ ID NO: 54 - protein, 22 aa, synthetic construct
  REGION 1..22: note = Description of Artificial Sequence: Synthetic peptide
LEGEGQGLEARNRELKERAESV

SEQ ID NO: 55 - protein, 22 aa, synthetic construct
  REGION 1..22: note = Description of Artificial Sequence: Synthetic peptide
LEGEAQGLEARNRELKERAESV

SEQ ID NO: 56 - protein, 22 aa, synthetic construct
  REGION 1..22: note = Description of Artificial Sequence: Synthetic peptide
LEGECQGLEARNRELKERAEAV

SEQ ID NO: 57 - protein, 22 aa, synthetic construct
  REGION 1..22: note = Description of Artificial Sequence: Synthetic peptide
LEGECQGLEARLRELKERAESV

SEQ ID NO: 58 - protein, 22 aa, synthetic construct
  REGION 1..22: note = Description of Artificial Sequence: Synthetic peptide
LEGECAGLEARNRELKERAESV

SEQ ID NO: 59 - protein, 22 aa, synthetic construct
  REGION 1..22: note = Description of Artificial Sequence: Synthetic peptide
LEGRCQGLRAENRELEERAESV

SEQ ID NO: 60 - protein, 22 aa, synthetic construct
  REGION 1..22: note = Description of Artificial Sequence: Synthetic peptide
LEGRCQGLRAELRELEERAEAV

SEQ ID NO: 61 - protein, 22 aa, synthetic construct
  REGION 1..22: note = Description of Artificial Sequence: Synthetic peptide
LEGRAQGLRAELRELEERAEAV

SEQ ID NO: 62 - protein, 22 aa, synthetic construct
  REGION 1..22: note = Description of Artificial Sequence: Synthetic peptide
LEGRLQGLRAELRELEERAEAV

SEQ ID NO: 63 - protein, 22 aa, synthetic construct
  REGION 1..22: note = Description of Artificial Sequence: Synthetic peptide
LEGRLAGLRAELRELEERAEAV

SEQ ID NO: 64 - protein, 22 aa, synthetic construct
  REGION 1..22: note = Description of Artificial Sequence: Synthetic peptide
LEGRAAGLRAELRELEERAEAV

SEQ ID NO: 65 - protein, 22 aa, synthetic construct
  REGION 1..22: note = Description of Artificial Sequence: Synthetic peptide
  SITE 1: note = D-valine
  SITE 2: note = D-alanine
  SITE 3: note = D-glutamic acid
  SITE 4: note = D-alanine
  SITE 5: note = D-arginine
  SITE 6: note = D-glutamic acid
  SITE 7: note = D-glutamic acid
  SITE 8: note = D-leucine
  SITE 9: note = D-glutamic acid
  SITE 10: note = D-arginine
  SITE 11: note = D-leucine
  SITE 12: note = D-glutamic acid
  SITE 13: note = D-alanine
  SITE 14: note = D-arginine
  SITE 15: note = D-leucine
  SITE 16: note = D-glycine
  SITE 17: note = D-glutamine
  SITE 18: note = D-alanine
  SITE 19: note = D-arginine
  SITE 20: note = D-glycine
  SITE 21: note = D-glutamic acid
  SITE 22: note = D-leucine
VAEAREELERLEARLGQARGEL

SEQ ID NO: 66-67 - skipped (2 entries)

SEQ ID NO: 68 - protein, 15 aa, synthetic construct
  REGION 1..15: note = Description of Artificial Sequence: Synthetic peptide
KRPAATKKAGQAKKK

SEQ ID NO: 69 - protein, 5 aa, synthetic construct
  REGION 1..5: note = Description of Artificial Sequence: Synthetic peptide
VPTLK

SEQ ID NO: 70 - protein, 5 aa, synthetic construct
  REGION 1..5: note = Description of Artificial Sequence: Synthetic peptide
KLPVM

SEQ ID NO: 71 - protein, 9 aa, synthetic construct
  REGION 1..9: note = Description of Artificial Sequence: Synthetic peptide
PAAKRVKLD

SEQ ID NO: 72 - protein, 5 aa, synthetic construct
  REGION 1..5: note = Description of Artificial Sequence: Synthetic peptide
GRGDS

SEQ ID NO: 73 - protein, 6 aa, synthetic construct
  REGION 1..6: note = Description of Artificial Sequence: Synthetic peptide
GRGDNP

SEQ ID NO: 74 - DNA, 22 bp, synthetic construct
  misc_feature 1..22: note = Description of Artificial Sequence: Synthetic primer
  source 1..22: mol_type = other DNA
atggatgatgatatcgccgcgc

SEQ ID NO: 75 - DNA, 22 bp, synthetic construct
  misc_feature 1..22: note = Description of Artificial Sequence: Synthetic primer
  source 1..22: mol_type = other DNA
gaagcatttgcggtggacgatg

SEQ ID NO: 76 - DNA, 15 bp, synthetic construct
  misc_feature 1..15: note = Description of Artificial Sequence: Synthetic primer
  source 1..15: mol_type = other DNA
atggcgcacgctggg

SEQ ID NO: 77 - DNA, 21 bp, synthetic construct
  misc_feature 1..21: note = Description of Artificial Sequence: Synthetic primer
  source 1..21: mol_type = other DNA
cttgtggcccagataggcacc

SEQ ID NO: 78 - DNA, 23 bp, synthetic construct
  misc_feature 1..23: note = Description of Artificial Sequence: Synthetic primer
  source 1..23: mol_type = other DNA
gcccagactcacatcaccaagtg

SEQ ID NO: 79 - DNA, 25 bp, synthetic construct
  misc_feature 1..25: note = Description of Artificial Sequence: Synthetic primer
  source 1..25: mol_type = other DNA
atgtttggcctcaaaagaaacgcgg

SEQ ID NO: 80 - DNA, 33 bp, synthetic construct
  misc_feature 1..33: note = Description of Artificial Sequence: Synthetic primer
  source 1..33: mol_type = other DNA
tcttattagatatgccaaaccagctcctactcc

SEQ ID NO: 81 - DNA, 20 bp, synthetic construct
  misc_feature 1..20: note = Description of Artificial Sequence: Synthetic primer
  source 1..20: mol_type = other DNA
atgtcactcctggcgaccct

SEQ ID NO: 82 - DNA, 19 bp, synthetic construct
  misc_feature 1..19: note = Description of Artificial Sequence: Synthetic primer
  source 1..19: mol_type = other DNA
gcagctacgggtcctctgg

SEQ ID NO: 83 - DNA, 16 bp, synthetic construct
  misc_feature 1..16: note = Description of Artificial Sequence: Synthetic primer
  source 1..16: mol_type = other DNA
atgcacctgcagcccg

SEQ ID NO: 84 - DNA, 17 bp, synthetic construct
  misc_feature 1..17: note = Description of Artificial Sequence: Synthetic primer
  source 1..17: mol_type = other DNA
cgcgcagttgcccatgg

SEQ ID NO: 85 - DNA, 18 bp, synthetic construct
  misc_feature 1..18: note = Description of Artificial Sequence: Synthetic primer
  source 1..18: mol_type = other DNA
atgggtgccccgacgttg

SEQ ID NO: 86 - DNA, 21 bp, synthetic construct
  misc_feature 1..21: note = Description of Artificial Sequence: Synthetic primer
  source 1..21: mol_type = other DNA
tcaatccatggcagccagctg

SEQ ID NO: 87 - protein, 12 aa, synthetic construct
  REGION 1..12: note = Description of Artificial Sequence: Synthetic peptide
  REGION 1..12: note = This region may encompass 7-12 residues
RRRRRRRRRRRR